European Patent Application EP 4 696 377 A2, published February 18, 2026. Title: 5HT AGONISTS FOR TREATING DISORDERS. Applicant: THE REGENTS OF THE UNIVERSITY OF CALIFORNIA. Application EP. The sequence listing filed with the application follows.

SEQUENCE LISTING (6 sequences)

SEQ ID NO: 1 - DNA, 15 bp, Danio rerio
  source 1..15: mol_type = unassigned DNA
ttcatgattttactc

SEQ ID NO: 2 - DNA, 15 bp, synthetic construct
  misc_feature 1..15: note = scn1Lab mutant
  source 1..15: mol_type = other DNA
ttcaggattttactc

SEQ ID NO: 3 - protein, 5 aa, Danio rerio
FMILL

SEQ ID NO: 4 - protein, 5 aa, synthetic construct
  REGION 1..5: note = scn1Lab mutant
FRILL

SEQ ID NO: 5-6 - skipped (2 entries)